European Patent Application EP 4 406 973 A1, published July 31, 2024. Title: ANTIBODIES AND USES THEREOF FOR THE TREATMENT OF INFECTIONS CAUSED BY ENVELOPED VIRUSES. Applicant: Fundacio Privada Institut de Recerca de la SIDA - Caixa. Application EP. The sequence listing filed with the application follows.

SEQUENCE LISTING (166 sequences)

SEQ ID NO: 1 - protein, 8 aa, synthetic construct
GYTFTDYF

SEQ ID NO: 2 - protein, 8 aa, synthetic construct
IYPGSGHI

SEQ ID NO: 3 - protein, 13 aa, synthetic construct
ARYSTLDYYVMDQ

SEQ ID NO: 4 - protein, 13 aa, synthetic construct
ARYSTLDYYVLDQ

SEQ ID NO: 5 - protein, 12 aa, synthetic construct
QTLFNSGTRKNY

SEQ ID NO: 6-7 - skipped (2 entries)

SEQ ID NO: 8 - protein, 8 aa, synthetic construct
KQSYNLLT

SEQ ID NO: 9 - protein, 25 aa, synthetic construct
QVQLTQSGPELVRPGASVRLSCKAS

SEQ ID NO: 10 - protein, 17 aa, synthetic construct
INWVKQRPGQGLEWIAR

SEQ ID NO: 11 - protein, 39 aa, synthetic construct
NYNEKFKGKAIKLTAEESSSTAYMELSSLTSEDSAVYFC

SEQ ID NO: 12 - protein, 11 aa, synthetic construct
WGQGTSVTVSS

SEQ ID NO: 13 - protein, 25 aa, synthetic construct [sequence omitted]

SEQ ID NO: 14 - protein, 17 aa, synthetic construct
MHWVRQAPGQGLEWMGR

SEQ ID NO: 15 - protein, 38 aa, synthetic construct
NYAQKFQGRVTMTRDTSSSTAYMELSRLRSDDTAVYYC

SEQ ID NO: 16 - protein, 38 aa, synthetic construct
NYAQKFQGRVTMTRDTSISTAYMELSRLRSDDTAVYYC

SEQ ID NO: 17 - protein, 11 aa, synthetic construct
WGQGTLVTVSS

SEQ ID NO: 18 - protein, 26 aa, synthetic construct
DIVMTQSPDSLAVSLGERATINCKSS

SEQ ID NO: 19 - protein, 17 aa, synthetic construct
LAWYQQKSGQAPKLLIY

SEQ ID NO: 20 - protein, 36 aa, synthetic construct
TRESGVPDRFTGSGSGTDFTLTISSLQAEDLAVYYC

SEQ ID NO: 21 - protein, 11 aa, synthetic construct
FGAGTKLELIK

SEQ ID NO: 22 - protein, 26 aa, synthetic construct
DIVMTQSPDSLAVSLGERATINCKSS

SEQ ID NO: 23 - skipped

SEQ ID NO: 24 - protein, 36 aa, synthetic construct
TRESGVPDRFSGSGSGTDFTLTISSLQAEDVAVYYC

SEQ ID NO: 25 - protein, 11 aa, synthetic construct
FGQGTKLELIK

SEQ ID NO: 26 - protein, 120 aa, synthetic construct
QVQLVQSGAEVKKPGASVKVSCKASGYTFTDYFMHWVRQAPGQGLEWMGRIYPGSGHINYAQKFQGRBTMTRDTSSSTAYMELSRLRSDDTAVYYCARYSTLDYYVMDQWGQGTLVTVSS

SEQ ID NO: 27 - protein, 120 aa, synthetic construct
QVQLVQSGAEVKKPGASVKVSCKASGYTFTDYFMHWVRQAPGQGLEWMGRIYPGSGHINYAQKFQGRBTMTRDTSISTAYMELSRLRSDDTAVYYCARYSTLDYYVLDQWGQGTLVTVSS

SEQ ID NO: 28 - protein, 120 aa, synthetic construct
QVQLVQSGAEVKKPGASVKVSCKASGYTFTDYFMHWVRQAPGQGLEWMGRIYPGSGHINYAQKFQGRBTMTRDTSISTAYMELSRLRSDDTAVYYCARYSTLDYYVMDQWGQGTLVTVSS

SEQ ID NO: 29 - protein, 113 aa, synthetic construct
DIVMTQSPDSLAVSLGERATINCKSSQTLFNSGTRKNYLAWYQQKPGQPPKLLIYWASTRESGVPDRFSGSGSGTDFTLTISSLQAEDVAVYYCKQSYNLLTFGQGTKLELIK

SEQ ID NO: 30 - protein, 113 aa, synthetic construct
DIVMTQSPDSLAVSLGERATINCKSSQTLFNSGTRKNYLAWYQQKPGQPPKLLIYFASTRESGVPDRFSGSGSGTDFTLTISSLQAEDVAVYYCKQSYNLLTFGQGTKLELIK

SEQ ID NO: 31 - protein, 108 aa, synthetic construct
QVQLTQSGPELVRPGASVRLSCKASGYTFTDYFINWVKQRPGQGLEWIARIYPGSGHINYNEKFKGKAIKLTAEESSSTAYMELSSLTSEDSAVYFCWGQGTSVTVSS

SEQ ID NO: 32 - protein, 113 aa, synthetic construct
DIVMTQSPDSLAVSLGERATINCKSSQTLFNSGTRKNYLAWYQQKSGQAPKLLIYWASTRESGVPDRFSGSGSGTDFTLTISSLQAEDVAVYYCKQSYNLLTFGAGTKLELIK

SEQ ID NO: 33 - protein, 13 aa, synthetic construct
ARYSTLDYYVMDQ

SEQ ID NO: 34-39 - skipped (6 entries)

SEQ ID NO: 40 - protein, 8 aa, synthetic construct
GYSFTTYY

SEQ ID NO: 41 - protein, 7 aa, synthetic construct
ISCYNGA

SEQ ID NO: 42 - protein, 7 aa, synthetic construct
ISAYNGA

SEQ ID NO: 43 - protein, 7 aa, synthetic construct
ISCYSGA

SEQ ID NO: 44 - protein, 9 aa, synthetic construct
ARKGGWIPF

SEQ ID NO: 45 - protein, 9 aa, synthetic construct
ARKGGFIPF

SEQ ID NO: 46 - protein, 12 aa, synthetic construct
QSVLNSSNQKNF

SEQ ID NO: 47 - protein, 12 aa, synthetic construct
QSVLSSSNQKNF

SEQ ID NO: 48-49 - skipped (2 entries)

SEQ ID NO: 50 - protein, 6 aa, synthetic construct
HQYLSS

SEQ ID NO: 51 - protein, 25 aa, synthetic construct
EVQLQQSGPEVVKTGASVKISCKAS

SEQ ID NO: 52 - protein, 17 aa, synthetic construct
MHWVKQSHGKSLEWIGY

SEQ ID NO: 53 - protein, 39 aa, synthetic construct
TNYNQKFKGKATFTLDTSSSTAYMQFDSLTSEDSAVYYC

SEQ ID NO: 54 - protein, 13 aa, synthetic construct
DYWGQGTTLTVSS

SEQ ID NO: 55 - protein, 25 aa, synthetic construct [sequence omitted]

SEQ ID NO: 56 - protein, 17 aa, synthetic construct
MHWVRQAPGQRLEWMGW

SEQ ID NO: 57 - protein, 39 aa, synthetic construct
TKYSQKFQGRVTITRDTSASTAYMELSSLRSEDTAVYYC

SEQ ID NO: 58 - protein, 39 aa, synthetic construct
TKYSQKFQGRVTITRDTSISTAYMELSSLRSEDTAVYYC

SEQ ID NO: 59 - protein, 13 aa, synthetic construct
DYWGQGTTVTVSS

SEQ ID NO: 60 - protein, 26 aa, synthetic construct
NIMMTQSPSSLAVSAGEKVTMTCKSS

SEQ ID NO: 61 - protein, 17 aa, synthetic construct
LAWYQQKPGQSPKLLIY

SEQ ID NO: 62 - protein, 36 aa, synthetic construct
TRESGVPERFTGSGSGTDFSLTISSVQAEDLAVYYC

SEQ ID NO: 63 - protein, 12 aa, synthetic construct
YTFGGGTKLEIK

SEQ ID NO: 64 - protein, 26 aa, synthetic construct
DIVMTQSPDSLAVSLGERATINCKSS

SEQ ID NO: 65 - protein, 17 aa, synthetic construct
LAWYQQKPGQPPKLLIY

SEQ ID NO: 66 - protein, 36 aa, synthetic construct; identical to SEQ ID NO: 24

SEQ ID NO: 67 - protein, 12 aa, synthetic construct
YTFGGGTKLEIK

SEQ ID NO: 68 - protein, 118 aa, synthetic construct
QVQLVQSGAEVKKPGASVKVSCKASGYSFTTYYMHWVRQAPGQRLEWMGWISCYNGATKYSQKFQGRVTITRDTSASTAYMELSSLRSEDTAVYYCARKGGWIPFDYWGQGTTVTVSS

SEQ ID NO: 69 - protein, 118 aa, synthetic construct
QVQLVQSGAEVKKPGASVKVSCKASGYSFTTYYMHWVRQAPGQRLEWMGWISAYSGATKYSQKFQGRVTITRDTSASTAYMELSSLRSEDTAVYYCARKGGFIPFDYWGQGTTVTVSS

SEQ ID NO: 70 - protein, 118 aa, synthetic construct
QVQLVQSGAEVKKPGASVKVSCKASGYSFTTYYMHWVRQAPGQRLEWMGWISAYSGATKYSQKFQGRVTITRDTSASTAYMELSSLRSEDTAVYYCARKGGWIPFDYWGQGTTVTVSS

SEQ ID NO: 71-76 - skipped (6 entries)

SEQ ID NO: 77 - protein, 112 aa, synthetic construct
DIVMTQSPDSLAVSLGERATINCKSSQSVLNSSNQKNFLAWYQQKPGQPPKLLIYWASTRESGVPDRFSGSGSGTDFTLTISSLQAEDVAVYYCHQYLSSYTFGGGTKLEIK

SEQ ID NO: 78 - protein, 112 aa, synthetic construct
DIVMTQSPDSLAVSLGERATINCKSSQSVLSSSNQKNFLAWYQQKPGQPPKLLIYFASTRESGVPDRFSGSGSGTDFTLTISSLQAEDVAVYYCHQYLSSYTFGGGTKLEIK

SEQ ID NO: 79 - skipped

SEQ ID NO: 80 - protein, 112 aa, synthetic construct
DIVMTQSPDSLAVSLGERATINCKSSQSVLSSSNQKNFLAWYQQKPGQPPKLLIYWASTRESGVPDRFSGSGSGTDFTLTISSLQAEDVAVYYCHQYLSSYTFGGGTKLEIK

SEQ ID NO: 81-85 - skipped (5 entries)

SEQ ID NO: 86 - protein, 118 aa, synthetic construct
EVQLQQSGPEVVKTGASVKISCKASGYSFTTYYMHWVKQSHGKSLEWIGYISCYNGATNYNQKFKGKATFTLDTSSSTAYMQFDSLTSEDSAVYYCARKGGWIPFDYWGQGTTLTVSS

SEQ ID NO: 87 - protein, 112 aa, synthetic construct
NIMMTQSPSSLAVSAGEKVTMTCKSSQSVLNSSNQKNFLAWYQQKPGQSPKLLIYWASTRESGVPERFTGSGSGTDFSLTISSVQAEDLAVYYCHQYLSSYTFGGGTKLEIK

SEQ ID NO: 88 - protein, 9 aa, synthetic construct
ARKGGWIPF

SEQ ID NO: 89 - protein, 8 aa, synthetic construct
GYTFSTYW

SEQ ID NO: 90 - protein, 8 aa, synthetic construct
IAPSDGYT

SEQ ID NO: 91 - protein, 13 aa, synthetic construct
GGFYDGYPDFFDF

SEQ ID NO: 92 - protein, 12 aa, synthetic construct
QSLLNSNTQRNY

SEQ ID NO: 93 - skipped

SEQ ID NO: 94 - protein, 9 aa, synthetic construct
QQHYSSPYT

SEQ ID NO: 95 - protein, 25 aa, synthetic construct
QVQLHQPGSELVRPGTSVKLSCKAS

SEQ ID NO: 96 - protein, 17 aa, synthetic construct
MNWIKRRPGQGLEWIGV

SEQ ID NO: 97 - protein, 40 aa, synthetic construct
KYNQKFRGKAALTVDTSSSTAYMQVSSLTSEDSAVYYCAR

SEQ ID NO: 98 - protein, 11 aa, synthetic construct
WGQGTTLAVSS

SEQ ID NO: 99 - protein, 25 aa, synthetic construct [sequence omitted]

SEQ ID NO: 100 - protein, 17 aa, synthetic construct
MHWVRQAPGQGLEWMGI

SEQ ID NO: 101 - protein, 40 aa, synthetic construct
SYAQKFQGRVTMTRDTSTSTVYMELSSLRSEDTAVYYCAR

SEQ ID NO: 102 - protein, 11 aa, synthetic construct
WGQGTTVTVSS

SEQ ID NO: 103 - protein, 26 aa, synthetic construct
DIVMTQSPSSLAVSVGQKVTMNCKPS

SEQ ID NO: 104 - protein, 17 aa, synthetic construct
LAWYQQKPGQSPKLLVY

SEQ ID NO: 105 - protein, 36 aa, synthetic construct
TREYGVPERFIGSGSGTDFTLTISSVQAEDLADYFC

SEQ ID NO: 106 - protein, 10 aa, synthetic construct
FGGGTKLEIK

SEQ ID NO: 107 - protein, 26 aa, synthetic construct
DIVMTQSPDSLAVSLGERATINCKSS

SEQ ID NO: 108 - protein, 17 aa, synthetic construct
LAWYQQKPGQPPKLLIY

SEQ ID NO: 109 - protein, 36 aa, synthetic construct
TRESGVPDRFSGSGSGTDFTLTISSLQAEDVACYYC

SEQ ID NO: 110 - protein, 10 aa, synthetic construct
FGQGTKLEIK

SEQ ID NO: 111 - protein, 122 aa, synthetic construct
QVQLVQSGAEVKKPGASVKVSCKASGYTFSTYWMHWVRQAPGQGLEWMGIIAPSDGYTSYAQKFQGRVTMTRDTSTSTVYMELSSLRSEDTAVYYCARGGFYDGYPDFFDFWGQGTTVTVSS

SEQ ID NO: 112 - protein, 113 aa, synthetic construct
DIVMTQSPDSLAVSLGERATINCKSSQSLLNSNTQRNYLAWYQQKPGQPPKLLIYFASTRESGVPDRFSGSGSGTDFTLTISSLQAEDVACYYCQQHYSSPYTFGQGTKLEIK

SEQ ID NO: 113 - protein, 122 aa, synthetic construct
QVQLHQPGSELVRPGTSVKLSCKASGYTFSTYWMNWIKRRPGQGLEWIGVIAPSDGYTKYNQKFRGKAALTVDTSSSTAYMQVSSLTSEDSAVYYCARGGFYDGYPDFFDFWGQGTTLAVSS

SEQ ID NO: 114 - protein, 113 aa, synthetic construct
DIVMTQSPSSLAVSVGQKVTMNCKPSQSLLNSNTQRNYLAWYQQKPGQSPKLLVYFASTREYGVPERFIGSGSGTDFTLTISSVQAEDLADYFCQQHYSSPYTFGGGTKLEIK

SEQ ID NO: 115 - protein, 13 aa, synthetic construct
GGFYDGYPDFFDF

SEQ ID NO: 116 - protein, 5 aa, synthetic construct
NYWMH

SEQ ID NO: 117 - protein, 17 aa, synthetic construct
RIDPNSAGTKYNDNFKN

SEQ ID NO: 118 - protein, 10 aa, synthetic construct
EDFDSRNFDV

SEQ ID NO: 119 - protein, 30 aa, synthetic construct
QVQLQQPGAELVKPGASVKLSCMASGYIFT

SEQ ID NO: 120 - protein, 14 aa, synthetic construct
WVKQRPGRGLEWIG

SEQ ID NO: 121 - protein, 32 aa, synthetic construct
KATLTVDKSSKTSYMQLNSLTSADSAVYFCAR

SEQ ID NO: 122 - protein, 11 aa, synthetic construct
WGTGTTVTVSS

SEQ ID NO: 123 - protein, 12 aa, synthetic construct
RATSSVSSSYLH

SEQ ID NO: 124 - protein, 7 aa, synthetic construct
STSNLAS

SEQ ID NO: 125 - protein, 9 aa, synthetic construct
QQYSGYPLT

SEQ ID NO: 126 - protein, 23 aa, synthetic construct
ENVLTQSPAIMSASPGEKITMTC

SEQ ID NO: 127 - protein, 15 aa, synthetic construct
WFQQKSGASPKPWIY

SEQ ID NO: 128 - protein, 32 aa, synthetic construct
GVPARFSGSGSGTSYSLTISSVEAEDAATYYC

SEQ ID NO: 129 - protein, 10 aa, synthetic construct
FGGGTKVEIK

SEQ ID NO: 130 - protein, 119 aa, synthetic construct
QVQLQQPGAELVKPGASVKLSCMASGYIFTNYWMHWVKQRPGRGLEWIGRIDPNSAGTKYNDNFKNKATLTVDKSSKTSYMQLNSLTSADSAVYFCAREDFDSRNFDVWGTGTTVTVSS

SEQ ID NO: 131 - protein, 108 aa, synthetic construct
ENVLTQSPAIMSASPGEKITMTCRATSSVSSSYLHWFQQKSGASPKPWIYSTSNLASGVPARFSGSGSGTSYSLTISSVEAEDAATYYCQQYSGYPLTFGGGTKVEIK

SEQ ID NO: 132 - protein, 10 aa, synthetic construct
EDFDSRNFDV

SEQ ID NO: 133 - protein, 5 aa, synthetic construct
NGYWN

SEQ ID NO: 134 - protein, 16 aa, synthetic construct
FINYSGSTYYNPSLKS

SEQ ID NO: 135 - protein, 10 aa, synthetic construct
GVYYARFFDV

SEQ ID NO: 136 - protein, 30 aa, synthetic construct
EVQLQESGPSLVKPSQTLSLTCSVTGDSIT

SEQ ID NO: 137 - protein, 14 aa, synthetic construct
WIRNFPGNELEYMG

SEQ ID NO: 138 - protein, 32 aa, synthetic construct
RISITRDTSKNQYYLQLNSVTTEDTATYYCVL

SEQ ID NO: 139 - protein, 11 aa, synthetic construct
WGAGTTVTVSS

SEQ ID NO: 140 - protein, 11 aa, synthetic construct
KASQNVDTNVA

SEQ ID NO: 141 - protein, 7 aa, synthetic construct
SASYRYS

SEQ ID NO: 142 - protein, 9 aa, synthetic construct
QQYNSYPIT

SEQ ID NO: 143 - protein, 23 aa, synthetic construct
DIVMTQSQKFMSTSVGDRVSVTC

SEQ ID NO: 144 - protein, 15 aa, synthetic construct
WYQQKPGQSPKALIY

SEQ ID NO: 145 - protein, 32 aa, synthetic construct
GVPDRFTGSGSGTDFTLTISNVQSEDLAEYFC

SEQ ID NO: 146 - protein, 10 aa, synthetic construct
FGSGTKLEIK

SEQ ID NO: 147 - protein, 118 aa, synthetic construct
EVQLQESGPSLVKPSQTLSLTCSVTGDSITNGYWNWIRNFPGNELEYMGFINYSGSTYYNPSLKSRISITRDTSKNQYYLQLNSVTTEDTATYYCVLGVYYARFFDVWGAGTTVTVSS

SEQ ID NO: 148 - protein, 107 aa, synthetic construct
DIVMTQSQKFMSTSVGDRVSVTCKASQNVDTNVAWYQQKPGQSPKALIYSASYRYSGVPDRFTGSGSGTDFTLTISNVQSEDLAEYFCQQYNSYPITFGSGTKLEIK

SEQ ID NO: 149 - protein, 10 aa, synthetic construct
GVYYARFFDV

SEQ ID NO: 150 - protein, 330 aa, synthetic construct
ASTKGPSVFPLAPSSKSTSGGTAALGCLVKDYFPEPVTVSWNSGALTSGVHTFPAVLQSSGLYSLSSVVTVPSSSLGTQTYICNVNHKPSNTKVDKRVEPKSCDKTHTCPPCPAPELLGGPSVFLFPPKPKDTLMISRTPEVTCVVVDVSHEDPEVKFNWYVDGVEVHNAKTKPREEQYNSTYRVVSVLTVLHQDWLNGKEYKCKVSNKALPAPIEKTISKAKGQPREPQVYTLPPSREEMTKNQVSLTCLVKGFYPSDIAVEWESNGQPENNYKTTPPVLDSDGSFFLYSKLTVDKSRWQQGNVFSCSVMHEALHNHYTQKSLSLSPGK

SEQ ID NO: 151 - protein, 107 aa, synthetic construct [sequence omitted]

SEQ ID NO: 152 - protein, 660 aa, synthetic construct
MGFLPKLLLLASFFPAGQASWGVSSPQDVQGVKGSCLLIPCIFSFPADVEVPDGITAIWYYDYSGQRQVVSHSADPKLVEARFRGRTEFMGNPEHRVCNLLLKDLQPEDSGSYNFRFEISEVNRWSDVKGTLVTVTEEPRVPTIASPVELLEGTEVDFNCSTPYVCLQEQVRLQWQGQDPARSVTFNSQKFEPTGVGHLETLHMAMSWQDHGRILRCQLSVANHRAQSEIHLQVKYAPKGVKILLSPSGRNILPGELVTLTCQVNSSYPAVSSIKWLKDGVRLQTKTGVLHLPQAAWSDAGVYTCQAENGVGSLVSPPISLHIFMAEVQVSPAGPILENQTVTLVCNTPNEAPSDLRYSWYKNHVLLEDAHSHTLRLHLATRADTGFYFCEVQNVHGSERSGPVSVVVNHPPLTPVLTAFLETQAGLVGILSRDKTHTCPPCPAPELLGGPSVFLFPPKPKDTLMISRTPEVTCVVVDVSHEDPEVKFNWYVDGVEVHNAKTKPREEQYNSTYRVVSVLTVLHQDWLNGKEYKCKVSNKALPAPIEKTISKAKGQPREPQVYTLPPSRDELTKNQVSLTCLVKGFYPSDIAVEWESNGQPENNYKTTPPVLDSDGSFFLYSKLTVDKSRWQQGNVFSCSVMHEALHNHYTQKSLSLSPGK

SEQ ID NO: 153 - protein, 115 aa, synthetic construct
SWGVSSPQDVQGVKGSCLLIPCIFSFPADVEVPDGITAIWYYDYSGQRQVVSHSADPKLVEARFRGRTEFMGNPEHRVCNLLLKDLQPEDSGSYNFRFEISEVNRWSDVKGTLVT

SEQ ID NO: 154 - protein, 94 aa, synthetic construct
RVPTIASPVELLEGTEVDFNCSTPYVCLQEQVRLQWQGQDPARSVTFNSQKFEPTGVGHLETLHMAMSWQDHGRILRCQLSVANHRAQSEIHLQ

SEQ ID NO: 155 - protein, 82 aa, synthetic construct
KGVKILLSPSGRNILPGELVTLTCQVNSSYPAVSSIKWLKDGVRLQTKTGVLHLPQAAWSDAGVYTCQAENGVGSLVSPPIS

SEQ ID NO: 156 - protein, 79 aa, synthetic construct
EVQVSPAGPILENQTVTLVCNTPNEAPSDLRYSWYKNHVLLEDAHSHTLRLHLATRADTGFYFCEVQNVHGSERSGPVS

SEQ ID NO: 157 - protein, 134 aa, synthetic construct
DKTHTCPPCPAPELLGGPSVFLFPPKPKDTLMISRTPEVTCVVVDVSHEDPEVKFNWYVDGVEVHNAKTKPREEQYNSTYRVVSVLTVLHQDWLNGKEYKCKVSNKALPAPIEKTISKAKGQPREPQVYTLPPS

SEQ ID NO: 158 - protein, 86 aa, synthetic construct
QVSLTCLVKGFYPSDIAVEWESNGQPENNYKTTPPVLDSDGSFFLYSKLTVDKSRWQQGNVFSCSVMHEALHNHYTQKSLSLSPGK

SEQ ID NO: 159 - protein, 5 aa, synthetic construct
GGGGS

SEQ ID NO: 160 - protein, 10 aa, synthetic construct
GGGGSGGGGS

SEQ ID NO: 161 - protein, 15 aa, synthetic construct
GGGGSGGGGSGGGGS

SEQ ID NO: 162 - protein, 5 aa, synthetic construct
EPKSS

SEQ ID NO: 163 - protein, 20 aa, synthetic construct
METDTLLLWVLLLWVPGSTG

SEQ ID NO: 164 - protein, 26 aa, synthetic construct
MATGSRTSLLLAFGLLCLPWLQEGSA

SEQ ID NO: 165 - protein, 641 aa, synthetic construct
SWGVSSPQDVQGVKGSCLLIPCIFSFPADVEVPDGITAIWYYDYSGQRQVVSHSADPKLVEARFRGRTEFMGNPEHRVCNLLLKDLQPEDSGSYNFRFEISEVNRWSDVKGTLVTVTEEPRVPTIASPVELLEGTEVDFNCSTPYVCLQEQVRLQWQGQDPARSVTFNSQKFEPTGVGHLETLHMAMSWQDHGRILRCQLSVANHRAQSEIHLQVKYAPKGVKILLSPSGRNILPGELVTLTCQVNSSYPAVSSIKWLKDGVRLQTKTGVLHLPQAAWSDAGVYTCQAENGVGSLVSPPISLHIFMAEVQVSPAGPILENQTVTLVCNTPNEAPSDLRYSWYKNHVLLEDAHSHTLRLHLATRADTGFYFCEVQNVHGSERSGPVSVVVNHPPLTPVLTAFLETQAGLVGILSRDKTHTCPPCPAPELLGGPSVFLFPPKPKDTLMISRTPEVTCVVVDVSHEDPEVKFNWYVDGVEVHNAKTKPREEQYNSTYRVVSVLTVLHQDWLNGKEYKCKVSNKALPAPIEKTISKAKGQPREPQVYTLPPSRDELTKNQVSLTCLVKGFYPSDIAVEWESNGQPENNYKTTPPVLDSDGSFFLYSKLTVDKSRWQQGNVFSCSVMHEALHNHYTQKSLSLSPGK

SEQ ID NO: 166 - protein, 227 aa, synthetic construct
DKTHTCPPCPAPELLGGPSVFLFPPKPKDTLMISRTPEVTCVVVDVSHEDPEVKFNWYVDGVEVHNAKTKPREEQYNSTYRVVSVLTVLHQDWLNGKEYKCKVSNKALPAPIEKTISKAKGQPREPQVYTLPPSRDELTKNQVSLTCLVKGFYPSDIAVEWESNGQPENNYKTTPPVLDSDGSFFLYSKLTVDKSRWQQGNVFSCSVMHEALHNHYTQKSLSLSPGK